European Patent Application EP 4 524 159 A1, published March 19, 2025. Title: 一种抗体及其用途. Applicant: 四川汇宇制药股份有限公司. The sequence listing filed with the application follows.

SEQUENCE LISTING (406 sequences)

SEQ ID NO: 1 - protein, 8 aa, synthetic construct
  source 1..8: note = IMGT 3B12H9/3B12H5 CDR-H1
GYSFTIYW

SEQ ID NO: 2 - protein, 8 aa, synthetic construct
  source 1..8: note = IMGT 3C11 CDR-H1
GYNFISYW

SEQ ID NO: 3 - protein, 8 aa, synthetic construct
  source 1..8: note = IMGT 5G9 CDR-H1
GYIFLNYW

SEQ ID NO: 4 - protein, 8 aa, synthetic construct
  source 1..8: note = IMGT 4E12G10/SB4/SB14 CDR-H1
GYTFTNYW

SEQ ID NO: 5 - protein, 8 aa, synthetic construct
  source 1..8: note = IMGT 6A7 CDR-H1
GYSFTSYW

SEQ ID NO: 6 - protein, 9 aa, synthetic construct
  source 1..9: note = IMGT 6G9/3F1A11 CDR-H1
GYSITSDYA

SEQ ID NO: 7 - protein, 9 aa, synthetic construct
  source 1..9: note = IMGT 20G4/27D11/3F1A11-H-12 CDR-H1
GYSITSGYY

SEQ ID NO: 8 - protein, 8 aa, synthetic construct
  source 1..8: note = IMGT 3A9 CDR-H1
GDSITTGY

SEQ ID NO: 9 - protein, 8 aa, synthetic construct
  source 1..8: note = IMGT 19F7D6 CDR-H1
GFTFSTYT

SEQ ID NO: 10 - protein, 8 aa, synthetic construct
  source 1..8: note = IMGT 3E7/SB2/SB15 CDR-H1
GFTFSSYT

SEQ ID NO: 11 - protein, 8 aa, synthetic construct
  source 1..8: note = IMGT 5B8/8C9 CDR-H1
GLTFTHYH

SEQ ID NO: 12 - protein, 8 aa, synthetic construct
  source 1..8: note = IMGT 4B7 CDR-H1
GLTFTYYH

SEQ ID NO: 13 - protein, 10 aa, synthetic construct
  source 1..10: note = IMGT 12E6/G10F6/14A10C5/1CP-064 CDR-H1
GFSLSTSGMG

SEQ ID NO: 14 - protein, 8 aa, synthetic construct
  source 1..8: note = IMGT 8E5 CDR-H1
GYTLTDFS

SEQ ID NO: 15 - protein, 8 aa, synthetic construct
  source 1..8: note = IMGT 27A3 CDR-H1
GYTFTYYS

SEQ ID NO: 16 - protein, 8 aa, synthetic construct
  source 1..8: note = IMGT 10D2 CDR-H1
GYTFTDYS

SEQ ID NO: 17 - protein, 8 aa, synthetic construct
  source 1..8: note = IMGT 24G4/1CP-065/1CP-068 CDR-H1
GFNIKDYY

SEQ ID NO: 18 - protein, 8 aa, synthetic construct
  source 1..8: note = IMGT 1CP-061 CDR-H1
GYTFTSYW

SEQ ID NO: 19 - protein, 8 aa, synthetic construct
  source 1..8: note = IMGT 1CP-063 CDR-H1
GYTFTSYY

SEQ ID NO: 20 - protein, 8 aa, synthetic construct
  source 1..8: note = IMGT 1CP-062 CDR-H1
GFSLTTYG

SEQ ID NO: 21 - protein, 8 aa, synthetic construct
  source 1..8: note = IMGT 1CP-067/1CP-069 CDR-H1
GFTFSVYG

SEQ ID NO: 22 - protein, 8 aa, synthetic construct
  source 1..8: note = IMGT 1CP-066 CDR-H1
GYAFTKYG

SEQ ID NO: 23 - protein, 8 aa, synthetic construct
  source 1..8: note = IMGT SB1 CDR-H1
GYTFTDHA

SEQ ID NO: 24 - protein, 8 aa, synthetic construct
  source 1..8: note = IMGT 3E7/SB2/SB15 CDR-H1
GFTFSSYT

SEQ ID NO: 25 - protein, 8 aa, synthetic construct
  source 1..8: note = IMGT SB3 CDR-H1
GFPFSSYT

SEQ ID NO: 26 - protein, 8 aa, synthetic construct
  source 1..8: note = IMGT 4E12G10/SB4/SB14 CDR-H1
GYTFTNYW

SEQ ID NO: 27 - protein, 8 aa, synthetic construct
  source 1..8: note = IMGT SB5 CDR-H1
GFSLTDFG

SEQ ID NO: 28 - protein, 8 aa, synthetic construct
  source 1..8: note = IMGT SB6 CDR-H1
GFTFNSSY

SEQ ID NO: 29 - protein, 8 aa, synthetic construct
  source 1..8: note = IMGT SB7 CDR-H1
GYTFTDYA

SEQ ID NO: 30 - protein, 10 aa, synthetic construct
  source 1..10: note = IMGT SB8 CDR-H1
GFSLSTSGVG

SEQ ID NO: 31 - protein, 8 aa, synthetic construct
  source 1..8: note = IMGT SB9 CDR-H1
GFTFSSFT

SEQ ID NO: 32 - protein, 9 aa, synthetic construct
  source 1..9: note = IMGT SB10/SB17 CDR-H1
GFSLSTSGM

SEQ ID NO: 33 - protein, 8 aa, synthetic construct
  source 1..8: note = IMGT SB11 CDR-H1
GFNIQDTY

SEQ ID NO: 34 - protein, 8 aa, synthetic construct
  source 1..8: note = IMGT SB12 CDR-H1
GYTFSRYW

SEQ ID NO: 35 - protein, 8 aa, synthetic construct
  source 1..8: note = IMGT SB13 CDR-H1
GFTFSDFY

SEQ ID NO: 36 - protein, 8 aa, synthetic construct
  source 1..8: note = IMGT SB16 CDR-H1
GYPFTDYA

SEQ ID NO: 37 - protein, 9 aa, synthetic construct
  source 1..9: note = IMGT SB18 CDR-H1
GFSLTTSGM

SEQ ID NO: 38 - protein, 8 aa, synthetic construct
  source 1..8: note = IMGT 3B12H9/3B12H5 CDR-H2
VYPGNDDT

SEQ ID NO: 39 - protein, 8 aa, synthetic construct
  source 1..8: note = IMGT 3C11/5G9 CDR-H2
IYPGNTDT

SEQ ID NO: 40 - protein, 8 aa, synthetic construct
  source 1..8: note = IMGT 4E12G10/SB4 CDR-H2
NYPGDNYR

SEQ ID NO: 41 - protein, 8 aa, synthetic construct
  source 1..8: note = IMGT 6A7 CDR-H2
IHPSDSET

SEQ ID NO: 42 - protein, 7 aa, synthetic construct
  source 1..7: note = IMGT 6G9 CDR-H2
IIYSGRT

SEQ ID NO: 43 - protein, 7 aa, synthetic construct
  source 1..7: note = IMGT 3F1A11 CDR-H2
ISYNTYT

SEQ ID NO: 44 - protein, 7 aa, synthetic construct
  source 1..7: note = IMGT 20G4/27D11/3F1A11-H-12 CDR-H2
ITYDDSH

SEQ ID NO: 45 - protein, 7 aa, synthetic construct
  source 1..7: note = IMGT 3A9 CDR-H2
ILYSGST

SEQ ID NO: 46 - protein, 8 aa, synthetic construct
  source 1..8: note = IMGT 19F7D6/SB2/SB3 CDR-H2
ISSGGIYT

SEQ ID NO: 47 - protein, 8 aa, synthetic construct
  source 1..8: note = IMGT 3E7 CDR-H2
ISNGGGNT

SEQ ID NO: 48 - protein, 10 aa, synthetic construct
  source 1..10: note = IMGT 5B8/4B7/8C9 CDR-H2
IRNKAYGYTT

SEQ ID NO: 49 - protein, 7 aa, synthetic construct
  source 1..7: note = IMGT 12E6/1CP-064 CDR-H2
IWWDDVK

SEQ ID NO: 50 - protein, 7 aa, synthetic construct
  source 1..7: note = IMGT G10F6/SB10 CDR-H2
IYWDDDK

SEQ ID NO: 51 - protein, 7 aa, synthetic construct
  source 1..7: note = IMGT 14A10C5 CDR-H2
IYWDDEK

SEQ ID NO: 52 - protein, 8 aa, synthetic construct
  source 1..8: note = IMGT 8E5 CDR-H2
INTETGAP

SEQ ID NO: 53 - protein, 8 aa, synthetic construct
  source 1..8: note = IMGT 27A3 CDR-H2
INTETGEP

SEQ ID NO: 54 - protein, 8 aa, synthetic construct
  source 1..8: note = IMGT 10D2 CDR-H2
INTETGQP

SEQ ID NO: 55 - protein, 8 aa, synthetic construct
  source 1..8: note = IMGT 24G4 CDR-H2
IDPENGDT

SEQ ID NO: 56 - protein, 8 aa, synthetic construct
  source 1..8: note = IMGT 1CP-061 CDR-H2
IYPSDSYT

SEQ ID NO: 57 - protein, 8 aa, synthetic construct
  source 1..8: note = IMGT 1CP-063 CDR-H2
IYPGNVNS

SEQ ID NO: 58 - protein, 7 aa, synthetic construct
  source 1..7: note = IMGT 1CP-062 CDR-H2
IWSDGNT

SEQ ID NO: 59 - protein, 8 aa, synthetic construct
  source 1..8: note = IMGT 1CP-067 CDR-H2
LSGGSNYT

SEQ ID NO: 60 - protein, 8 aa, synthetic construct
  source 1..8: note = IMGT 1CP-069 CDR-H2
LSGGDNYT

SEQ ID NO: 61 - protein, 8 aa, synthetic construct
  source 1..8: note = IMGT 1CP-066 CDR-H2
INTYTGEA

SEQ ID NO: 62 - protein, 8 aa, synthetic construct
  source 1..8: note = IMGT 1CP-065 CDR-H2
IDPENDNT

SEQ ID NO: 63 - protein, 8 aa, synthetic construct
  source 1..8: note = IMGT 1CP-068 CDR-H2
IDPENGNT

SEQ ID NO: 64 - protein, 8 aa, synthetic construct
  source 1..8: note = IMGT SB1 CDR-H2
ISFSYDNT

SEQ ID NO: 65 - protein, 8 aa, synthetic construct
  source 1..8: note = IMGT 19F7D6/SB2/SB3 CDR-H2
ISSGGIYT

SEQ ID NO: 66 - protein, 8 aa, synthetic construct
  source 1..8: note = IMGT 4E12G10/SB4 CDR-H2
NYPGDNYR

SEQ ID NO: 67 - protein, 7 aa, synthetic construct
  source 1..7: note = IMGT SB5 CDR-H2
IWANGRI

SEQ ID NO: 68 - protein, 8 aa, synthetic construct
  source 1..8: note = IMGT SB6 CDR-H2
IFAGTGGT

SEQ ID NO: 69 - protein, 8 aa, synthetic construct
  source 1..8: note = IMGT SB7 CDR-H2
KSVYYGIT

SEQ ID NO: 70 - protein, 7 aa, synthetic construct
  source 1..7: note = IMGT SB8 CDR-H2
IWWDDEK

SEQ ID NO: 71 - protein, 8 aa, synthetic construct
  source 1..8: note = IMGT SB9 CDR-H2
ISSSGSYT

SEQ ID NO: 72 - protein, 7 aa, synthetic construct
  source 1..7: note = IMGT G10F6/SB10 CDR-H2
IYWDDDK

SEQ ID NO: 73 - protein, 8 aa, synthetic construct
  source 1..8: note = IMGT SB11 CDR-H2
IDPANDNT

SEQ ID NO: 74 - protein, 8 aa, synthetic construct
  source 1..8: note = IMGT SB12 CDR-H2
ILPGSDFT

SEQ ID NO: 75 - protein, 10 aa, synthetic construct
  source 1..10: note = IMGT SB13 CDR-H2
SRDKTNDYTT

SEQ ID NO: 76 - protein, 8 aa, synthetic construct
  source 1..8: note = IMGT SB14 CDR-H2
IFPGTGTT

SEQ ID NO: 77 - protein, 8 aa, synthetic construct
  source 1..8: note = IMGT SB15 CDR-H2
ISGGINYT

SEQ ID NO: 78 - protein, 8 aa, synthetic construct
  source 1..8: note = IMGT SB16 CDR-H2
IAPYSDNT

SEQ ID NO: 79 - protein, 7 aa, synthetic construct
  source 1..7: note = IMGT SB17/SB18 CDR-H2
IWWNDDK

SEQ ID NO: 80 - protein, 11 aa, synthetic construct
  source 1..11: note = IMGT 3B12H9/3B12H5 CDR-H3
TRHTYDEVFDY

SEQ ID NO: 81 - protein, 11 aa, synthetic construct
  source 1..11: note = IMGT 3C11/5G9 CDR-H3
IRYDYDRGMDY

SEQ ID NO: 82 - protein, 13 aa, synthetic construct
  source 1..13: note = IMGT 4E12G10 CDR-H3
TRSGGTRYYTMDY

SEQ ID NO: 83 - protein, 13 aa, synthetic construct
  source 1..13: note = IMGT 6A7 CDR-H3
TINYESFYYAMDY

SEQ ID NO: 84 - protein, 15 aa, synthetic construct
  source 1..15: note = IMGT 6G9 CDR-H3
AREDYYGGSYGGLDY

SEQ ID NO: 85 - protein, 13 aa, synthetic construct
  source 1..13: note = IMGT 3F1A11 CDR-H3
AGGDYYGTGAVDY

SEQ ID NO: 86 - protein, 15 aa, synthetic construct
  source 1..15: note = IMGT 20G4/27D11/3F1A11-H-12 CDR-H3
ARGNYYANYPHAMDY

SEQ ID NO: 87 - protein, 10 aa, synthetic construct
  source 1..10: note = IMGT 3A9 CDR-H3
ARGDYGAMDY

SEQ ID NO: 88 - protein, 15 aa, synthetic construct
  source 1..15: note = IMGT 19F7D6/SB2/SB3 CDR-H3
SSPHSYAISYGYFDY

SEQ ID NO: 89 - protein, 14 aa, synthetic construct
  source 1..14: note = IMGT 3E7 CDR-H3
ASSYGNYRGAWFAY

SEQ ID NO: 90 - protein, 14 aa, synthetic construct
  source 1..14: note = IMGT 5B8/8C9 CDR-H3
VREGGYGYDGTFAY

SEQ ID NO: 91 - protein, 14 aa, synthetic construct
  source 1..14: note = IMGT 4B7 CDR-H3
AREGGYGYDGTFAY

SEQ ID NO: 92 - protein, 16 aa, synthetic construct
  source 1..16: note = IMGT 12E6 CDR-H3
ARIDHGYGSNYWDFDV

SEQ ID NO: 93 - protein, 14 aa, synthetic construct
  source 1..14: note = IMGT G10F6 CDR-H3
ARVPGNWDEDAMDY

SEQ ID NO: 94 - protein, 13 aa, synthetic construct
  source 1..13: note = IMGT 14A10C5 CDR-H3
AREGSANWEAMDY

SEQ ID NO: 95 - protein, 12 aa, synthetic construct
  source 1..12: note = IMGT 8E5 CDR-H3
SRGRDYDPHFDY

SEQ ID NO: 96 - protein, 6 aa, synthetic construct
  source 1..6: note = IMGT 27A3 CDR-H3
ANAMDY

SEQ ID NO: 97 - protein, 12 aa, synthetic construct
  source 1..12: note = IMGT 10D2 CDR-H3
TRTFYYDYVGDY

SEQ ID NO: 98 - protein, 11 aa, synthetic construct
  source 1..11: note = IMGT 24G4 CDR-H3
NPCGTGPWFAY

SEQ ID NO: 99 - protein, 13 aa, synthetic construct
  source 1..13: note = IMGT 1CP-061 CDR-H3
TRCLRRRDWYFDV

SEQ ID NO: 100 - protein, 13 aa, synthetic construct
  source 1..13: note = IMGT 1CP-063 CDR-H3
AREDYGHYYAMDY

SEQ ID NO: 101 - protein, 13 aa, synthetic construct
  source 1..13: note = IMGT 1CP-062 CDR-H3
AKNYRNYDYAMDY

SEQ ID NO: 102 - protein, 13 aa, synthetic construct
  source 1..13: note = IMGT 1CP-067/1CP-069 CDR-H3
ATEDGLIGTWGDY

SEQ ID NO: 103 - protein, 12 aa, synthetic construct
  source 1..12: note = IMGT 1CP-064 CDR-H3
ARMGGKVPWFAY

SEQ ID NO: 104 - protein, 15 aa, synthetic construct
  source 1..15: note = IMGT 1CP-066 CDR-H3
SRGDDYGTGGYVLFY

SEQ ID NO: 105 - protein, 13 aa, synthetic construct
  source 1..13: note = IMGT 1CP-065 CDR-H3
ARFYGSYYYAMDY

SEQ ID NO: 106 - protein, 9 aa, synthetic construct
  source 1..9: note = IMGT 1CP-068 CDR-H3
AGRLYAMEY

SEQ ID NO: 107 - protein, 14 aa, synthetic construct
  source 1..14: note = IMGT SB1 CDR-H3
ARDCYGSNRGYFDY

SEQ ID NO: 108 - protein, 15 aa, synthetic construct
  source 1..15: note = IMGT 19F7D6/SB2/SB3 CDR-H3
SSPHSYAISYGYFDY

SEQ ID NO: 109 - protein, 13 aa, synthetic construct
  source 1..13: note = IMGT SB4 CDR-H3
TRSGGSRYYTMDY

SEQ ID NO: 110 - protein, 13 aa, synthetic construct
  source 1..13: note = IMGT SB5 CDR-H3
ARDHDYDVEAMDY

SEQ ID NO: 111 - protein, 9 aa, synthetic construct
  source 1..9: note = IMGT SB6 CDR-H3
ARHGLGYDY

SEQ ID NO: 112 - protein, 14 aa, synthetic construct
  source 1..14: note = IMGT SB7 CDR-H3
ARDSYGSSRGYFDY

SEQ ID NO: 113 - protein, 9 aa, synthetic construct
  source 1..9: note = IMGT SB8 CDR-H3
VKEGDGMDY

SEQ ID NO: 114 - protein, 15 aa, synthetic construct
  source 1..15: note = IMGT SB9 CDR-H3
TSPDYYGRSYGYFDY

SEQ ID NO: 115 - protein, 13 aa, synthetic construct
  source 1..13: note = IMGT SB10 CDR-H3
TREGSADWEALDY

SEQ ID NO: 116 - protein, 11 aa, synthetic construct
  source 1..11: note = IMGT SB11 CDR-H3
AREDAYPWFAY

SEQ ID NO: 117 - protein, 15 aa, synthetic construct
  source 1..15: note = IMGT SB12 CDR-H3
ARKDYYGNYDYAMDY

SEQ ID NO: 118 - protein, 16 aa, synthetic construct
  source 1..16: note = IMGT SB13 CDR-H3
ARDGVYYYGSSYTLDY

SEQ ID NO: 119 - protein, 12 aa, synthetic construct
  source 1..12: note = IMGT SB14 CDR-H3
ARTNWEGYYFDY

SEQ ID NO: 120 - protein, 15 aa, synthetic construct
  source 1..15: note = IMGT SB15 CDR-H3
ARHDRYDGYYYVMDY

SEQ ID NO: 121 - protein, 13 aa, synthetic construct
  source 1..13: note = IMGT SB16 CDR-H3
AAYGNYGYYTMDY

SEQ ID NO: 122 - protein, 14 aa, synthetic construct
  source 1..14: note = IMGT SB17 CDR-H3
ARIGYYYGTYALDY

SEQ ID NO: 123 - protein, 10 aa, synthetic construct
  source 1..10: note = IMGT SB18 CDR-H3
ARLRDGGFAY

SEQ ID NO: 124 - protein, 11 aa, synthetic construct
  source 1..11: note = IMGT 3B12H9/27A3/SB9 CDR-L1
QSLLDSDGKTY

SEQ ID NO: 125 - protein, 6 aa, synthetic construct
  source 1..6: note = IMGT 3B12H5/3C11 CDR-L1
EDIYYR

SEQ ID NO: 126 - protein, 5 aa, synthetic construct
  source 1..5: note = IMGT 5G9/24G4/1CP-068/SB17 CDR-L1
SSVSY

SEQ ID NO: 127 - protein, 11 aa, synthetic construct
  source 1..11: note = IMGT 4E12G10/1CP-067/1CP-069 CDR-L1
KSLLHSNGITY

SEQ ID NO: 128 - protein, 10 aa, synthetic construct
  source 1..10: note = IMGT 6A7 CDR-L1
KSVSTSGYSY

SEQ ID NO: 129 - protein, 11 aa, synthetic construct
  source 1..11: note = IMGT 6G9 CDR-L1
QSIVHSNGNTY

SEQ ID NO: 130 - protein, 11 aa, synthetic construct
  source 1..11: note = IMGT 3F1A11/3F1A11-H-12 CDR-L1
QTLVHTNGNTY

SEQ ID NO: 131 - protein, 10 aa, synthetic construct
  source 1..10: note = IMGT 20G4 CDR-L1
ESVDHNGISF

SEQ ID NO: 132 - protein, 10 aa, synthetic construct
  source 1..10: note = IMGT 27D11 CDR-L1
ESVDNSGISF

SEQ ID NO: 133 - protein, 11 aa, synthetic construct
  source 1..11: note = IMGT 3A9 CDR-L1
QSIVHSNGKTY

SEQ ID NO: 134 - protein, 11 aa, synthetic construct
  source 1..11: note = IMGT 19F7D6/SB2 CDR-L1
QSLLDIDGKTY

SEQ ID NO: 135 - protein, 12 aa, synthetic construct
  source 1..12: note = IMGT 3E7 CDR-L1
QSLLYSNNQRNY

SEQ ID NO: 136 - protein, 10 aa, synthetic construct
  source 1..10: note = IMGT 5B8/4B7/8C9 CDR-L1
ESVDNYGISF

SEQ ID NO: 137 - protein, 11 aa, synthetic construct
  source 1..11: note = IMGT 12E6 CDR-L1
KSLLHSDGKTY

SEQ ID NO: 138 - protein, 11 aa, synthetic construct
  source 1..11: note = IMGT G10F6 CDR-L1
QNIVHTNGNTY

SEQ ID NO: 139 - protein, 11 aa, synthetic construct
  source 1..11: note = IMGT 14A10C5 CDR-L1
QNIVYTNGITY

SEQ ID NO: 140 - protein, 6 aa, synthetic construct
  source 1..6: note = IMGT 8E5 CDR-L1
QSISDF

SEQ ID NO: 141 - protein, 6 aa, synthetic construct
  source 1..6: note = IMGT 10D2/1CP-065 CDR-L1
QDVSTA

SEQ ID NO: 142 - protein, 10 aa, synthetic construct
  source 1..10: note = IMGT 1CP-061 CDR-L1
ESVDYSGYSF

SEQ ID NO: 143 - protein, 6 aa, synthetic construct
  source 1..6: note = IMGT 1CP-063 CDR-L1
QDIKSY

SEQ ID NO: 144 - protein, 10 aa, synthetic construct
  source 1..10: note = IMGT 1CP-062/1CP-064 CDR-L1
ESVDSYGNSF

SEQ ID NO: 145 - protein, 6 aa, synthetic construct
  source 1..6: note = IMGT 1CP-066 CDR-L1
ENIYNN

SEQ ID NO: 146 - protein, 6 aa, synthetic construct
  source 1..6: note = IMGT SB1 CDR-L1
QDINRF

SEQ ID NO: 147 - protein, 11 aa, synthetic construct
  source 1..11: note = IMGT 19F7D6/SB2 CDR-L1
QSLLDIDGKTY

SEQ ID NO: 148 - protein, 11 aa, synthetic construct
  source 1..11: note = IMGT SB3 CDR-L1
QSLLDFDGKTY

SEQ ID NO: 149 - protein, 11 aa, synthetic construct
  source 1..11: note = IMGT SB4 CDR-L1
RSLLHNNGITY

SEQ ID NO: 150 - protein, 5 aa, synthetic construct
  source 1..5: note = IMGT SB5 CDR-L1
SSVIY

SEQ ID NO: 151 - protein, 6 aa, synthetic construct
  source 1..6: note = IMGT SB6 CDR-L1
QSVNTD

SEQ ID NO: 152 - protein, 6 aa, synthetic construct
  source 1..6: note = IMGT SB7 CDR-L1
QDINSF

SEQ ID NO: 153 - protein, 9 aa, synthetic construct
  source 1..9: note = IMGT SB8 CDR-L1
TGAVATSNY

SEQ ID NO: 154 - protein, 11 aa, synthetic construct
  source 1..11: note = IMGT 3B12H9/27A3/SB9 CDR-L1
QSLLDSDGKTY

SEQ ID NO: 155 - protein, 11 aa, synthetic construct
  source 1..11: note = IMGT SB10 CDR-L1
QTIVYSNGNSY

SEQ ID NO: 156 - protein, 10 aa, synthetic construct
  source 1..10: note = IMGT SB11 CDR-L1
QSVSTSSYSY

SEQ ID NO: 157 - protein, 6 aa, synthetic construct
  source 1..6: note = IMGT SB12 CDR-L1
KSIGKY

SEQ ID NO: 158 - protein, 6 aa, synthetic construct
  source 1..6: note = IMGT SB13 CDR-L1
QDVSSS

SEQ ID NO: 159 - protein, 7 aa, synthetic construct
  source 1..7: note = IMGT SB14 CDR-L1
SSVRSSY

SEQ ID NO: 160 - protein, 6 aa, synthetic construct
  source 1..6: note = IMGT SB15 CDR-L1
QEISGY

SEQ ID NO: 161 - protein, 6 aa, synthetic construct
  source 1..6: note = IMGT SB16 CDR-L1
QDITNY

SEQ ID NO: 162 - protein, 5 aa, synthetic construct
  source 1..5: note = IMGT 5G9/24G4/1CP-068/SB17 CDR-L1
SSVSY

SEQ ID NO: 163 - protein, 6 aa, synthetic construct
  source 1..6: note = IMGT SB18 CDR-L1
QAISNY

SEQ ID NO: 164-196 - skipped (33 entries)

SEQ ID NO: 197 - protein, 9 aa, synthetic construct
  source 1..9: note = IMGT 3B12H9 CDR-L3
WQGTHFPWT

SEQ ID NO: 198 - protein, 9 aa, synthetic construct
  source 1..9: note = IMGT 3B12H5 CDR-L3
QHYWNTPWT

SEQ ID NO: 199 - protein, 9 aa, synthetic construct
  source 1..9: note = IMGT/Kabat/AbM/Chothia 3C11 CDR-L3
QHYWNIPWT

SEQ ID NO: 200 - protein, 9 aa, synthetic construct
  source 1..9: note = IMGT 5G9 CDR-L3
QQYHSYPYT

SEQ ID NO: 201 - protein, 9 aa, synthetic construct
  source 1..9: note = IMGT 4E12G10/SB4 CDR-L3
AQNLDLPYT

SEQ ID NO: 202 - protein, 9 aa, synthetic construct
  source 1..9: note = IMGT 6A7 CDR-L3
LHSRELPYT

SEQ ID NO: 203 - protein, 9 aa, synthetic construct
  source 1..9: note = IMGT 6G9/3F1A11/3F1A11-H-12/3A9 CDR-L3
FQGSHVPWT

SEQ ID NO: 204 - protein, 9 aa, synthetic construct
  source 1..9: note = IMGT 20G4/27D11 CDR-L3
QQNKEVPWT

SEQ ID NO: 205 - protein, 9 aa, synthetic construct
  source 1..9: note = IMGT 19F7D6/SB2/SB9 CDR-L3
WQGTHFPYT

SEQ ID NO: 206 - protein, 9 aa, synthetic construct
  source 1..9: note = IMGT 3E7 CDR-L3
QQYYSYPWT

SEQ ID NO: 207 - protein, 9 aa, synthetic construct
  source 1..9: note = IMGT/Kabat/AbM/Chothia 5B8/4B7/8C9 CDR-L3
QQSKEVPRT

SEQ ID NO: 208 - protein, 9 aa, synthetic construct
  source 1..9: note = IMGT 12E6 CDR-L3
MQHLEYPFT

SEQ ID NO: 209 - protein, 9 aa, synthetic construct
  source 1..9: note = IMGT G10F6 CDR-L3
FQGSHVPYT

SEQ ID NO: 210 - protein, 9 aa, synthetic construct
  source 1..9: note = IMGT 14A10C5/SB10 CDR-L3
FQSSHVPWT

SEQ ID NO: 211 - protein, 9 aa, synthetic construct
  source 1..9: note = IMGT/Kabat/AbM/Chothia 8E5 CDR-L3
QSAHSFPYT

SEQ ID NO: 212 - protein, 9 aa, synthetic construct
  source 1..9: note = IMGT 27A3 CDR-L3
WQGTHFPHT

SEQ ID NO: 213 - protein, 9 aa, synthetic construct
  source 1..9: note = IMGT 10D2 CDR-L3
QQHSSTPYT

SEQ ID NO: 214 - protein, 9 aa, synthetic construct
  source 1..9: note = IMGT 24G4 CDR-L3
QQWNSSPFT

SEQ ID NO: 215 - protein, 9 aa, synthetic construct
  source 1..9: note = IMGT 1CP-061/1CP-062 CDR-L3
QQSNEDPYT

SEQ ID NO: 216 - protein, 9 aa, synthetic construct
  source 1..9: note = IMGT 1CP-063 CDR-L3
LQYGESPWT

SEQ ID NO: 217 - protein, 9 aa, synthetic construct
  source 1..9: note = IMGT 1CP-067/1CP-069 CDR-L3
AQNLELPFT

SEQ ID NO: 218 - protein, 9 aa, synthetic construct
  source 1..9: note = IMGT 1CP-064 CDR-L3
QQNNEDPWT

SEQ ID NO: 219 - protein, 9 aa, synthetic construct
  source 1..9: note = IMGT 1CP-066 CDR-L3
QHFWGTPPT

SEQ ID NO: 220 - protein, 9 aa, synthetic construct
  source 1..9: note = IMGT 1CP-065 CDR-L3
QQHYSTPYT

SEQ ID NO: 221 - protein, 9 aa, synthetic construct
  source 1..9: note = IMGT 1CP-068 CDR-L3
QQWSSDPFT

SEQ ID NO: 222 - protein, 9 aa, synthetic construct
  source 1..9: note = IMGT SB1/SB7 CDR-L3
LQYDEFPRT

SEQ ID NO: 223 - protein, 9 aa, synthetic construct
  source 1..9: note = IMGT 19F7D6/SB2/SB9 CDR-L3
WQGTHFPYT

SEQ ID NO: 224 - protein, 9 aa, synthetic construct
  source 1..9: note = IMGT SB3 CDR-L3
WQGTHFPFT

SEQ ID NO: 225 - protein, 9 aa, synthetic construct
  source 1..9: note = IMGT 4E12G10/SB4 CDR-L3
AQNLDLPYT

SEQ ID NO: 226 - protein, 9 aa, synthetic construct
  source 1..9: note = IMGT SB5 CDR-L3
QQWSSYPPT

SEQ ID NO: 227 - protein, 10 aa, synthetic construct
  source 1..10: note = IMGT SB6 CDR-L3
QQDHSSPPWT

SEQ ID NO: 228 - protein, 9 aa, synthetic construct
  source 1..9: note = IMGT SB8 CDR-L3
ALWYSNHWV

SEQ ID NO: 229 - protein, 9 aa, synthetic construct
  source 1..9: note = IMGT 19F7D6/SB2/SB9 CDR-L3
WQGTHFPYT

SEQ ID NO: 230 - protein, 9 aa, synthetic construct
  source 1..9: note = IMGT 14A10C5/SB10 CDR-L3
FQSSHVPWT

SEQ ID NO: 231 - protein, 9 aa, synthetic construct
  source 1..9: note = IMGT SB11 CDR-L3
QHNWEIPWT

SEQ ID NO: 232 - protein, 9 aa, synthetic construct
  source 1..9: note = IMGT SB12 CDR-L3
QQHDEYPWT

SEQ ID NO: 233 - protein, 9 aa, synthetic construct
  source 1..9: note = IMGT SB13 CDR-L3
QQHYNTPPT

SEQ ID NO: 234 - protein, 10 aa, synthetic construct
  source 1..10: note = IMGT SB14 CDR-L3
QQYSGSPSWT

SEQ ID NO: 235 - protein, 9 aa, synthetic construct
  source 1..9: note = IMGT SB15 CDR-L3
LQYASYPYT

SEQ ID NO: 236 - protein, 9 aa, synthetic construct
  source 1..9: note = IMGT SB16 CDR-L3
QQGNTLPWT

SEQ ID NO: 237 - protein, 9 aa, synthetic construct
  source 1..9: note = IMGT SB17 CDR-L3
QQWSSYPLT

SEQ ID NO: 238 - protein, 9 aa, synthetic construct
  source 1..9: note = IMGT SB18 CDR-L3
QQYSKIPWT

SEQ ID NO: 239 - protein, 118 aa, synthetic construct
  source 1..118: note; note (original language) = 3B12H9/3B12H5重链可变区
EVQLQQSGTVLARPGASVKMSCKASGYSFTIYWVHWVKQRPGQGLEWIGAVYPGNDDTSYNQNFKGKAKLTAVTSATTAYMELSSLTIDDSAVYYCTRHTYDEVFDYWGQGTTVTVSS

SEQ ID NO: 240 - protein, 118 aa, synthetic construct
  source 1..118: note; note (original language) = 3C11重链可变区
EVQLQQSGTVLARPGASVKMSCKASGYNFISYWLHWIKQRPGQGLEWIGGIYPGNTDTTYNQKFKGKAKVTAVTSATTAYMELSSLTNEDSAVYYCIRYDYDRGMDYWGQGTTVTVSS

SEQ ID NO: 241 - protein, 118 aa, synthetic construct
  source 1..118: note; note (original language) = 5G9重链可变区
EVQLQQSGTVLARPGASVKMSCKASGYIFLNYWMHWVKQRPGQGLEWIGGIYPGNTDTTYNQKFKGKAKVTAVTSATTAYMELSSLTNEDSAVYYCIRYDYDRGMDYWGQGTTVTVSS

SEQ ID NO: 242 - protein, 120 aa, synthetic construct
  source 1..120: note; note (original language) = 4E12G10重链可变区
EVQLQQSGAELVRPGTSVKISCKASGYTFTNYWLGWVKQRPGHGLEWIGDNYPGDNYRNFNEKFKGKATLTTDASSSTAYLQLSSLISEDSAVYFCTRSGGTRYYTMDYWGQGTTVTVSS

SEQ ID NO: 243 - protein, 120 aa, synthetic construct
  source 1..120: note; note (original language) = 6A7重链可变区
EVQLKESGAELVRPGASVKVSCKASGYSFTSYWMNWVKQRPGQGLEWIGMIHPSDSETKLNQKFRDRASLTVDKSSSTAYMQLSSPTSEDSAVYYCTINYESFYYAMDYWGQGTTVTVSS

SEQ ID NO: 244 - protein, 122 aa, synthetic construct
  source 1..122: note; note (original language) = 6G9重链可变区
EVQLKESGPGLVKPSQSLSLTCTVTGYSITSDYAWNWIRQFPGNKLEWMGYIIYSGRTSYNPSLKSRISITRDTSKNQFFLQLNSVTTEDTATYYCAREDYYGGSYGGLDYWGQGTTVTVSS

SEQ ID NO: 245 - protein, 120 aa, synthetic construct
  source 1..120: note; note (original language) = 3F1A11重链可变区
EVKLVESGPGLVKPSQSLSLTCTVTGYSITSDYAWNWIRQFPGNKLEWMGYISYNTYTSYNPSLKSRISVTRDTSKNQFFLQLKSVTIEDTATYFCAGGDYYGTGAVDYWGQGTTVTVSS

SEQ ID NO: 246 - protein, 122 aa, synthetic construct
  source 1..122: note; note (original language) = 20G4重链可变区
EVQLKESGPGLVKPSQSLSLTCSVTGYSITSGYYWNWIRQFPGNKLDWMGYITYDDSHYYNPSLKDRLSITRDTSKNQFFLKLNSVTAEDTATYFCARGNYYANYPHAMDYWGQGTTVTVSS

SEQ ID NO: 247 - protein, 122 aa, synthetic construct
  source 1..122: note; note (original language) = 27D11重链可变区
EVTLKESGPGLVKPSQSLSLTCSVTGYSITSGYYWNWIRQFPGNKLDWMGYITYDDSHYYNPSLKHRLSITRDTSKNQFFLKLNSVTAEDTATYFCARGNYYANYPHAMDYWGQGTTVTVSS

SEQ ID NO: 248 - protein, 122 aa, synthetic construct
  source 1..122: note; note (original language) = 3F1A11-H-12重链可变区
EVKLVESGPGLVKPSQSLSLTCSVTGYSITSGYYWNWIRQFPGNKLDWMGYITYDDSHYYNPSLKDRLSITRDTSKNQFFLKLNSVTAEDTATYFCARGNYYANYPHAMDYWGQGTTVTVSS

SEQ ID NO: 249 - protein, 116 aa, synthetic construct
  source 1..116: note; note (original language) = 3A9重链可变区
EVKLVESGSSLVKPSQTLSLTCSVTGDSITTGYWNWIRKFPGNKLEYMGYILYSGSTYYNPSLKSRISITRDTSKNQYYLQLNSVTTEDTATYYCARGDYGAMDYWGQGTTVTVSS

SEQ ID NO: 250 - protein, 122 aa, synthetic construct
  source 1..122: note; note (original language) = 19F7D6重链可变区
EVKLVESGGGLVKPGGSLKLSCAASGFTFSTYTMSWVRQTPEKRLEWVATISSGGIYTYYPDSVKGRFTISRDNAKDTLYLQMSSLRSEDTAVYYCSSPHSYAISYGYFDYWGQGTTVTVSS

SEQ ID NO: 251 - protein, 121 aa, synthetic construct
  source 1..121: note; note (original language) = 3E7重链可变区
EVQLKESGGGLVQPGGSLQLSCAASGFTFSSYTMSWVRQTLEKRLEWVAYISNGGGNTYYPDTLKGRFTISRDNAKNILYLQLSSLKSEDTAMYYCASSYGNYRGAWFAYWGQGTTVTVSS

SEQ ID NO: 252 - protein, 123 aa, synthetic construct
  source 1..123: note; note (original language) = 5B8重链可变区
EVQLKESGGGLVQPGGSLRISCATSGLTFTHYHMSWVRQPPGKAPEWLAIIRNKAYGYTTDYSASVRGRFTISRDDSQSILYLQMNTLRAEDSATYYCVREGGYGYDGTFAYWGQGTTVTVSS

SEQ ID NO: 253 - protein, 123 aa, synthetic construct
  source 1..123: note; note (original language) = 4B7重链可变区
EVQLQQSGGGLVQPGGSLRLSCATSGLTFTYYHMSWVRQPPGKAPEWLAIIRNKAYGYTTEYSASVKGRFTISRDDSQSILYLQMNTLRTEDSATYYCAREGGYGYDGTFAYWGQGTTVTVSS

SEQ ID NO: 254 - protein, 123 aa, synthetic construct
  source 1..123: note; note (original language) = 8C9重链可变区
EVQLKESGGGLVQPGGSLRISCATSGLTFTHYHMSWVRQPPGKAPEWLAIIRNKAYGYTTDYSASVRGRFTISRDDSQSILYLQMNTLRPEDSATYYCVREGGYGYDGTFAYWGQGTTVTVSS

SEQ ID NO: 255 - protein, 124 aa, synthetic construct
  source 1..124: note; note (original language) = 12E6重链可变区
EVQLKESGPGILQPSQTLSLTCSFSGFSLSTSGMGVGWIRQPSGKGLEWLAHIWWDDVKLYNPALKSRLTISKETSNNQVFLKIASVDAADTATYYCARIDHGYGSNYWDFDVWGAGTTVTVSS

SEQ ID NO: 256 - protein, 122 aa, synthetic construct
  source 1..122: note; note (original language) = G10F6重链可变区
EVKLVESGPGILQPSQTLSLTCSFSGFSLSTSGMGVSWVRQPSGKGLEWLAHIYWDDDKRYNPSLKGRLTISKDTPRNQVFLEITSVDTTDTATYYCARVPGNWDEDAMDYWGQGTTVTVSS

SEQ ID NO: 257 - protein, 121 aa, synthetic construct
  source 1..121: note; note (original language) = 14A10C5重链可变区
EVKLVESGPGILQPSQTLSLTCSFSGFSLSTSGMGVSWIRQPSGKGLEWLAHIYWDDEKRYNPSLKSRLTISKDTSSNQVFLKITSVDTADTATYYCAREGSANWEAMDYWGQGTTVTVSS

SEQ ID NO: 258 - protein, 119 aa, synthetic construct
  source 1..119: note; note (original language) = 8E5重链可变区
EVQLKESGPELKKPGETVKISCKASGYTLTDFSMHWLKQAPGKGLKWMGWINTETGAPTYADDFKGRFALSLDTSANTAYLQINNLKNEDTATYFCSRGRDYDPHFDYWGQGTTVTVSS

SEQ ID NO: 259 - protein, 113 aa, synthetic construct
  source 1..113: note; note (original language) = 27A3重链可变区
EVQLKESGPELKKPGETVKISCKASGYTFTYYSMHWVKQTPGKGLKWMGWINTETGEPTYADDFKGRFAFSLETSDSTAYLQINNLKNEDTATYFCANAMDYWGQGTTVTVSS

SEQ ID NO: 260 - protein, 119 aa, synthetic construct
  source 1..119: note; note (original language) = 10D2重链可变区
EVQLQQSGPELKKPGETVKISCKASGYTFTDYSMHWVKQAPGKGLKWMGWINTETGQPTYADDFKGRFAFSLETSASSAYLQINNLKNEDTATYFCTRTFYYDYVGDYWGQGTTVTVSS

SEQ ID NO: 261 - protein, 118 aa, synthetic construct
  source 1..118: note; note (original language) = 24G4重链可变区
EVQLKESGAELVRSGASVKLSCTASGFNIKDYYIHWVKQRPEQGLEWIGWIDPENGDTEYVPKFQGKATLTADTSSNTAYLQLNSLTSEDTAVYYCNPCGTGPWFAYWGQGTTVTVSS

SEQ ID NO: 262 - protein, 120 aa, synthetic construct
  source 1..120: note; note (original language) = 1CP-061重链可变区
EVQLKESGAELVRPGASVKLSCKASGYTFTSYWINWVRQRPGQGLEWIGNIYPSDSYTNYNQKFKDKATLTVDKSSSTAYMQLSSPTSEDSAVYYCTRCLRRRDWYFDVWGQGTTVTVSS

SEQ ID NO: 263 - protein, 120 aa, synthetic construct
  source 1..120: note; note (original language) = 1CP-063重链可变区
EVNLKESGPELVKPGASVRISCKASGYTFTSYYIHWVKQRPGQGLEWIGWIYPGNVNSKYNEKFKGKVTLTADKSSITAYMQLSSLTSEDSAVYFCAREDYGHYYAMDYWGQGTTVTVSS

SEQ ID NO: 264 - protein, 119 aa, synthetic construct
  source 1..119: note; note (original language) = 1CP-062重链可变区
EVKLVESGPGLVAPSQSLSITCTVSGFSLTTYGVHWVRQPPGKGLEWLVVIWSDGNTTYNSALKSRLSINKDNSKSQVFLKMNSLQTDDTAMYYCAKNYRNYDYAMDYWGQGTTVTVSS

SEQ ID NO: 265 - protein, 120 aa, synthetic construct
  source 1..120: note; note (original language) = 1CP-067重链可变区
EVQLKESGGGLVKPGGSLKLSCTASGFTFSVYGMSWVRQTPEKRLEWVATLSGGSNYTYYSDSVKGRFTISRDTGKNNLYLQMSSLSSDDTALYYCATEDGLIGTWGDYWGQGTTVTVSS

SEQ ID NO: 266 - protein, 120 aa, synthetic construct
  source 1..120: note; note (original language) = 1CP-069重链可变区
EVQLQQSGGGLVKPGGSLKLSCTASGFTFSVYGMSWVRQTPEKRLEWVATLSGGDNYTYYTDSVKGRFTISRDTAKNNLYLQMSSLRSEDTALYFCATEDGLIGTWGDYWGQGTTVTVSS

SEQ ID NO: 267 - protein, 120 aa, synthetic construct
  source 1..120: note; note (original language) = 1CP-064重链可变区
EVKLVESGPGILQPSQTLSLTCSFSGFSLSTSGMGVGWIRQPSGKGLEWLAHIWWDDVKRYNPALKSRLTISKDTSSSQVFLKIASVDTADTATYYCARMGGKVPWFAYWGQGTTVTVSS

SEQ ID NO: 268 - protein, 122 aa, synthetic construct
  source 1..122: note; note (original language) = 1CP-066重链可变区
EVTLKESGPELKKPGETVKISCKASGYAFTKYGMNWVKQAPGKDLKFMGWINTYTGEATYADDFKGRFDFSLEASASTAFLRINNLKNEDTATYFCSRGDDYGTGGYVLFYWGQGTTVTVSS

SEQ ID NO: 269 - protein, 120 aa, synthetic construct
  source 1..120: note; note (original language) = 1CP-065重链可变区
EVTLKESGAELVRPGALVKLSCKASGFNIKDYYMHWVKQRPEQGLEWIGWIDPENDNTIYDPKFQGKASITADTSSNTAYLQLSSLTSEDTAVYYCARFYGSYYYAMDYWGQGTTVTVSS

SEQ ID NO: 270 - protein, 116 aa, synthetic construct
  source 1..116: note; note (original language) = 1CP-068重链可变区
EVQLKESGAELVRPGALVKLSCKASGFNIKDYYMYWVKQRPEQGLEWIGWIDPENGNTIYDPKLQGKARITADTSSNTAYLQLSSLTSEDTAVYYCAGRLYAMEYWGQGTTVTVSS

SEQ ID NO: 271 - protein, 121 aa, synthetic construct
  source 1..121: note; note (original language) = SB1重链可变区
QVQLQQSGPDLVRPGESVKISCKGSGYTFTDHAIHWVRQSHAKSLEWIGVISFSYDNTKYNQNFKGKATMTVDKSSNTAYMELARLTSEDSAIYYCARDCYGSNRGYFDYWGQGTTLTVSS

SEQ ID NO: 272 - protein, 122 aa, synthetic construct
  source 1..122: note; note (original language) = SB2重链可变区
DVKLVESGGGLVKPGGSLKLSCAASGFTFSSYTMSWVRQTPEKRLEWVATISSGGIYTYYPDSVKGRFTISRDNAKDTLYLQMNSLRSEDTAVYYCSSPHSYAISYGYFDYWGQGTTLTVSS

SEQ ID NO: 273 - protein, 122 aa, synthetic construct
  source 1..122: note; note (original language) = SB3重链可变区
DVKLVESGGGLVEPGGSLKLSCAASGFPFSSYTMSWVRQTPEKRLEWVATISSGGIYTYYPDSVKGRFTISRDNAKDTLYLQMSSLRSEDTAVYYCSSPHSYAISYGYFDYWGQGTTLTVSS

SEQ ID NO: 274 - protein, 120 aa, synthetic construct
  source 1..120: note; note (original language) = SB4重链可变区
QVQLQQSGAELVRPGTSVKISCKASGYTFTNYWLGWVKQRPGHGLEWIGDNYPGDNYRNFNEKFKGKATLTTDASSSTAYLQLSSLISEDSAVYFCTRSGGSRYYTMDYWGQGTSVTVSS

SEQ ID NO: 275 - protein, 119 aa, synthetic construct
  source 1..119: note; note (original language) = SB5重链可变区
QVQLRESGPGLVAPSQSLSITCTVSGFSLTDFGVNWVRQPPGKGLEWLGIIWANGRIEYNSALKSRLSISKDNSRSQVFLKLNSLQTDDTARYYCARDHDYDVEAMDYWGQGTSVTVSA

SEQ ID NO: 276 - protein, 116 aa, synthetic construct
  source 1..116: note; note (original language) = SB6重链可变区
QGQMQQSGAELVKPGASVKLSCKTSGFTFNSSYITWLKQKPGQSLEWIAWIFAGTGGTYYNEKFTDKAQLTVDTTSSTAYMQFSSLTTEDSAIYYCARHGLGYDYWGQGTTLTVSS

SEQ ID NO: 277 - protein, 121 aa, synthetic construct
  source 1..121: note; note (original language) = SB7重链可变区
QVQLQQSGPELVSPGESVKISCKGSGYTFTDYAVHWVKQSHSKSLEWIGVKSVYYGITKYSQNFKDKATMTVDKSSSTAYMELARLTSEDSAIYYCARDSYGSSRGYFDYWGQGTTLTVSS

SEQ ID NO: 278 - protein, 117 aa, synthetic construct
  source 1..117: note; note (original language) = SB8重链可变区
QVTLKESGPGILKPSQTLSLTCSFSGFSLSTSGVGVGWIRQPSGKGLEWLAHIWWDDEKYYNPSLKSHFTISKDTSRNQVFLKITSVDTADTATYYCVKEGDGMDYWGQGTSVTVSS

SEQ ID NO: 279 - protein, 122 aa, synthetic construct
  source 1..122: note; note (original language) = SB9重链可变区
DVKLVESGGGLVKPGGSLKLSCAASGFTFSSFTMSWVRQTPEKRLEWVATISSSGSYTYYPDSVKGRFTISRDNAKNTLYLQMSSLKSEDTAMYYCTSPDYYGRSYGYFDYWGQGTTLTVSS

SEQ ID NO: 280 - protein, 121 aa, synthetic construct
  source 1..121: note; note (original language) = SB10重链可变区
QVTLKESGPGILQPSQTLSLTCSFSGFSLSTSGMGVSWFRQPSGKGLEWLAHIYWDDDKRYNPSLKSRLTISKDTSSNQVFLRITNVDTSDTATYYCTREGSADWEALDYWGQGTSVTVSS

SEQ ID NO: 281 - protein, 118 aa, synthetic construct
  source 1..118: note; note (original language) = SB11重链可变区
EVQLQQSGAELVKPGASVKLSCTASGFNIQDTYILWVKQRPEQGLEWIGGIDPANDNTNYGPNFQGKATITADTSSNTAYLQLSSLTSEDSAVYYCAREDAYPWFAYWGQGTLVTVSS

SEQ ID NO: 282 - protein, 122 aa, synthetic construct
  source 1..122: note; note (original language) = SB12重链可变区
QVQLQQSGAELMKPGASVKISCKATGYTFSRYWVEWVKQRPGHGLEWIGDILPGSDFTNYNEKFKGKATFTADSSSNTAYMQLSSLTSEDSAVYYCARKDYYGNYDYAMDYWGQGTSVTVSS

SEQ ID NO: 283 - protein, 125 aa, synthetic construct
  source 1..125: note; note (original language) = SB13重链可变区
EVKLVESGGGLVQPGGSLRLSCATSGFTFSDFYMEWVRQPPGKRLEWIAVSRDKTNDYTTEYSASMKGRFIVSRDTSQSILYLQMNALRAEDTAIYYCARDGVYYYGSSYTLDYWGQGTSVTVSS

SEQ ID NO: 284 - protein, 119 aa, synthetic construct
  source 1..119: note; note (original language) = SB14重链可变区
QVQLQQSGNEVVKPGASVKLSCKTSGYTFTNYWLQWVKQRPGQGLEWIGEIFPGTGTTYYNEKFKDQATVTIDTSSSTAYIHLSSLTSEDSAVYFCARTNWEGYYFDYWGQGTTLTVSS

SEQ ID NO: 285 - protein, 122 aa, synthetic construct
  source 1..122: note; note (original language) = SB15重链可变区
EVKLVESGGGLVKPGGSLKLSCAASGFTFSSYGMSWVRQTPEKRLEWVATISGGINYTYYRDSVEGRFTISRDNAKNNLYLQMSRLRSEDTALYYCARHDRYDGYYYVMDYWGQGTSVTVSS

SEQ ID NO: 286 - protein, 120 aa, synthetic construct
  source 1..120: note; note (original language) = SB16重链可变区
QVQLQQSGPELVRPGVSVRISCKGSGYPFTDYAIHWVKQGHGKNLEWIGVIAPYSDNTGYNQRFKGKATMTVDKSSSTAYMELARLTSEDSAIYYCAAYGNYGYYTMDYWGQGTSVTVSS

SEQ ID NO: 287 - protein, 122 aa, synthetic construct
  source 1..122: note; note (original language) = SB17重链可变区
QVTLKESGPGILQPSQTLSLTCSFSGFSLSTSGMSVGWIRQPSGKGLEWLAHIWWNDDKYYNPALKTRLTISKDSSNNQIFLKIASVVTADSATYYCARIGYYYGTYALDYWGPGTSVTVSS

SEQ ID NO: 288 - protein, 118 aa, synthetic construct
  source 1..118: note; note (original language) = SB18重链可变区
QVTLKESGPGILQPSQTLSLTCSFSGFSLTTSGMNVGWLRQPSGKGLEWLAHIWWNDDKHSNPVLKSRLTISKDTSNNQAFLKIANVVTADSATYYCARLRDGGFAYWGQGTLVTVSA

SEQ ID NO: 289 - protein, 112 aa, synthetic construct
  source 1..112: note; note (original language) = 3B12H9轻链可变区
EIVLTQSPLTLSVTIGQPASISCKSSQSLLDSDGKTYLNWLLQRPGQSPKRLIYLVSKLDSGVPDRFTGSGSGTDFTLKISRVEAEDLGVYYCWQGTHFPWTFGGGTKLEIK

SEQ ID NO: 290 - protein, 107 aa, synthetic construct
  source 1..107: note; note (original language) = 3B12H5轻链可变区
DIVMTQSPSSLSVSLGDRVTITCKASEDIYYRLAWYQQKPGNAPRLLISGGTNLEAGIPSRFSGSGSGKDYTLSITSLQTEDVAIYYCQHYWNTPWTFGGGTKLEIK

SEQ ID NO: 291 - protein, 107 aa, synthetic construct
  source 1..107: note; note (original language) = 3C11轻链可变区
DIQMTQSPSSFSVSLGDRVTITCRASEDIYYRLAWYQQKPGNAPRLLISGATALETGVPSRFSGSGSGKDYTLSITSLQTEDVATYYCQHYWNIPWTFGGGTKLEIK

SEQ ID NO: 292 - protein, 106 aa, synthetic construct
  source 1..106: note; note (original language) = 5G9轻链可变区
DIVMTQAPAIMSASPGEKVTISCSASSSVSYIYWYQQKPGSSPKPWIYRTSNLASGVPARFSGSGSGTSYSLTISSMEAEDAATYYCQQYHSYPYTFGGGTKLEIK

SEQ ID NO: 293 - protein, 112 aa, synthetic construct
  source 1..112: note; note (original language) = 4E12G10轻链可变区
DIVMTQAAFSNPVTLGTSASISCRSSKSLLHSNGITYLYWYLQKPGQSPQLLIYQMSNLASGVPDRFSSSGSGTDFTLSISRVEAGDVGVYYCAQNLDLPYTFGGGTKLEIK

SEQ ID NO: 294 - protein, 111 aa, synthetic construct
  source 1..111: note; note (original language) = 6A7轻链可变区
DIVMTQSPASLAVSLGQRATISCRASKSVSTSGYSYMHWYQQKPGQPPKLLLYLASNLESGVPARFSGSGSGADFTLNIHPVEEEDAATYYCLHSRELPYTFGGGTKLEIK

SEQ ID NO: 295 - protein, 112 aa, synthetic construct
  source 1..112: note; note (original language) = 6G9轻链可变区
DIVMTQSPLSLPVSLGDQASISCRSSQSIVHSNGNTYLEWYLQKPGQSPKLLIYKVSNRFSGVPDRFSGSGSGTDFTLKISRVEAEDLGVYYCFQGSHVPWTFGGGTKLEIK

SEQ ID NO: 296 - protein, 112 aa, synthetic construct
  source 1..112: note; note (original language) = 3F1A11/3F1A11-H-12轻链可变区
EIVLTQSPLSLPVSLGDQASISCRSRQTLVHTNGNTYLDWYLQKPGQSPKLLIYKVSIRFSGVPDRFSGSRSGTDFTLKISRVEAEDLGIYYCFQGSHVPWTFGGGTKLEIK

SEQ ID NO: 297 - protein, 111 aa, synthetic construct
  source 1..111: note; note (original language) = 20G4轻链可变区
EIVITQSPASLAVSLGQRASISCRASESVDHNGISFMNWFQQKPGQPPKLLIYAASNQGSGVPARFSGSGSRTDFSLSIHPMEEDDTAIYFCQQNKEVPWTFGGGTKLEIK

SEQ ID NO: 298 - protein, 111 aa, synthetic construct
  source 1..111: note; note (original language) = 27D11轻链可变区
DIVMTQSPASLAVSLGQRATISCRASESVDNSGISFMNWFQQKPGQPPKLLIYAASNQGSGVPARFSGSGSRTDFSLSIHPMEEDDTAMYFCQQNKEVPWTFGGGTKLEIK

SEQ ID NO: 299 - protein, 112 aa, synthetic construct
  source 1..112: note; note (original language) = 3A9轻链可变区
DIQMTQSPLSLPVSLGDQASISCRSGQSIVHSNGKTYLEWYLQKPGQSPKLLIYKVSTRFSGVPDRFSGSGSGTDFTLKITRVEAEDLGVYYCFQGSHVPWTFGGGTKLEIK

SEQ ID NO: 300 - protein, 112 aa, synthetic construct
  source 1..112: note; note (original language) = 19F7D6轻链可变区
DIVMTQSPLTLSITIGQPASISCRSSQSLLDIDGKTYLNWLLQRPGQSPKRLIYLVSELDSGVPDRFTGSGSGTDFTLKISGVEAEDLGIYYCWQGTHFPYTFGGGTKLEIK

SEQ ID NO: 301 - protein, 113 aa, synthetic construct
  source 1..113: note; note (original language) = 3E7轻链可变区
DIQMTQSPSSLAVSVGEKVSMSCKSSQSLLYSNNQRNYLAWYQQKPGQSPKLLIYWASTWESGVPDRFTGSGSGTAFTLTISSVKAEDLAVYYCQQYYSYPWTFGGGTKLEIK

SEQ ID NO: 302 - protein, 111 aa, synthetic construct
  source 1..111: note; note (original language) = 5B8轻链可变区
EIVLTQSPASLAVSLGQRATISCRASESVDNYGISFMSWFQQKPGQPPKLLIYAASNQGSGVPDRFSGSGSGTDFSLNIHPMEEDDTAMYFCQQSKEVPRTFGGGTKLEIK

SEQ ID NO: 303 - protein, 111 aa, synthetic construct
  source 1..111: note; note (original language) = 4B7轻链可变区
DVVMTQTPASLAVSLGQRATISCRASESVDNYGISFMNWFQQKPGQPPKLLIYAASNQGSGVPARFSGSGSGTDFSLNIHPMEEDDTAMYFCQQSKEVPRTFGGGTKLEIK

SEQ ID NO: 304 - protein, 111 aa, synthetic construct
  source 1..111: note; note (original language) = 8C9轻链可变区
DIQMTQSPASLAVSLGQRATISCRASESVDNYGISFMNWFQQKPGQPPKLLIYAASNQGSGVPDRFSGSGSGTDFSLNIHPMEEDDTAMYFCQQSKEVPRTFGGGTKLEIK

SEQ ID NO: 305 - protein, 112 aa, synthetic construct
  source 1..112: note; note (original language) = 12E6轻链可变区
DIVMTQAAPSVPVTPGGSVSISCRSTKSLLHSDGKTYLYWFLQRPGQSPQLLIYRMSNLASGVPDRFSGSGSGTAFTLRISRVEAEDVGVYYCMQHLEYPFTFGSGTKLEIK

SEQ ID NO: 306 - protein, 112 aa, synthetic construct
  source 1..112: note; note (original language) = G10F6轻链可变区
DIQMTQSPLSLPVSLGDQASISCRSSQNIVHTNGNTYLEWYLQKVGQSPKLLIYKVSNRFSGVPDRFSGSGSGTDFTLKISRVEAEDLGVYYCFQGSHVPYTFGGGTKLEIK

SEQ ID NO: 307 - protein, 112 aa, synthetic construct
  source 1..112: note; note (original language) = 14A10C5轻链可变区
DIVMTQAALSLPVSLGDQASISCRSSQNIVYTNGITYLEWYLQKPGQSPKLLIYKVSNRFSGVPDRFSGSGSATDFTLKISRVEAEDLGVYYCFQSSHVPWTFGGGTKLEIK

SEQ ID NO: 308 - protein, 107 aa, synthetic construct
  source 1..107: note; note (original language) = 8E5轻链可变区
EIVLTQSPATLSVTPGDRVSLSCRASQSISDFLHWYQQRSHESPRLLIKYASQSISGIPSRFGGSGSGSDFTLNINTVEPEDVGMYYCQSAHSFPYTFGGGTKLEIK

SEQ ID NO: 309 - protein, 112 aa, synthetic construct
  source 1..112: note; note (original language) = 27A3轻链可变区
DIVMTQTPLTLSVTIGQPASISCKSSQSLLDSDGKTYLNWLLQRPGQSPKRLIYLVSKLDSGVPDRFTGSGSGTDFTLKISRVEAEDLGVYYCWQGTHFPHTFGGGTKLEIK

SEQ ID NO: 310 - protein, 107 aa, synthetic construct
  source 1..107: note; note (original language) = 10D2轻链可变区
DIVMTQSHKFMSTSVGDRVSITCKASQDVSTAVAWYRQKPGQSPKLLIYWASTRHTGVPDRLTGSGSGTDFALTINSVQAEDLALYYCQQHSSTPYTFGGGTKLEIK

SEQ ID NO: 311 - protein, 106 aa, synthetic construct
  source 1..106: note; note (original language) = 24G4轻链可变区
DIQMTQSPAILSASPGEKVTMTCRASSSVSYIHWYQQKPGSSPDPWIYATSFLASGVPGRFSGSGSGTSYSLTISRLEAEDAATYYCQQWNSSPFTFGGGTKLEIK

SEQ ID NO: 312 - protein, 111 aa, synthetic construct
  source 1..111: note; note (original language) = 1CP-061轻链可变区
DVVMTQTPASLAVSLGQRATISCRASESVDYSGYSFMHWYQQKPGQPPKLLIYRASNLESGIPARFSGSGSRTDFTLTINPVEADDVATYYCQQSNEDPYTFGGGTKLEIK

SEQ ID NO: 313 - protein, 107 aa, synthetic construct
  source 1..107: note; note (original language) = 1CP-063轻链可变区
DIVMTQSPSSMYASLGERVTITCKASQDIKSYLSWYQQKPWKSPKTLIYYATSLADGVPSRFSGSGSGQDYSLTISSLESDDTATYYCLQYGESPWTFGGGTKLEIK

SEQ ID NO: 314 - protein, 111 aa, synthetic construct
  source 1..111: note; note (original language) = 1CP-062轻链可变区
DIVMTQTPASLAVSLGQRATISCRASESVDSYGNSFMHWYQQKPGQPPKLLIYRASNLESGIPARFSGSGSRTDFTLTINPVEADDVATYYCQQSNEDPYTFGGGTKLEIK

SEQ ID NO: 315 - protein, 112 aa, synthetic construct
  source 1..112: note; note (original language) = 1CP-067轻链可变区
DIVMTQAAFSNPVTLGTSASISCRSTKSLLHSNGITYLYWFLQKPGQSPQLLIYQMSNLASGVPDRFSSSGSGTDFTLRISRVEAEDVGVYYCAQNLELPFTFGGGTKLEIK

SEQ ID NO: 316 - protein, 112 aa, synthetic construct
  source 1..112: note; note (original language) = 1CP-069轻链可变区
DIVMTQAAFSNPVTLGTSASISCRSTKSLLHSNGITYLYWYLQKPGQSPQLLIYQMSNLASGVPDRFSSSGSGTDFTLRISRVEAEDVGVYYCAQNLELPFTFGGGTKLEIK

SEQ ID NO: 317 - protein, 111 aa, synthetic construct
  source 1..111: note; note (original language) = 1CP-064轻链可变区
DVVMTQTPASLAVSLGQRATISCRASESVDSYGNSFMHWYQQKPGQPPKLLIYLASNLESGVPARFSGSGSRTDFTLTIDPVEADDAATYYCQQNNEDPWTFGGGTKLEIK

SEQ ID NO: 318 - protein, 107 aa, synthetic construct
  source 1..107: note; note (original language) = 1CP-066轻链可变区
DIVMTQAAASLSVTVGETVTITCRASENIYNNLAWYQQQQGKSPQLLVYAATNLADGVPSRFSGSGSGTHYSLKINSLQSEDFGFYYCQHFWGTPPTFGGGTKLEIK

SEQ ID NO: 319 - protein, 107 aa, synthetic construct
  source 1..107: note; note (original language) = 1CP-065轻链可变区
DIVMTQSPKFMSTSVGDRVSITCKASQDVSTAVTWYQQKPGQSPKLLIYWASTRHTGVPDRFTGSGSGTDYTLTISSVQAEDLALYYCQQHYSTPYTFGGGTKLEIK

SEQ ID NO: 320 - protein, 106 aa, synthetic construct
  source 1..106: note; note (original language) = 1CP-068轻链可变区
DVVMTQTPALMSASPGEKVTMTCSASSSVSYMYWYQQKPRSSPKPWIYLTSNLASGVPARFSGSGSGTSYSLTISSMEAEDAATYYCQQWSSDPFTFGGGTKLEIK

SEQ ID NO: 321 - protein, 107 aa, synthetic construct
  source 1..107: note; note (original language) = SB1轻链可变区
DIRMTQSPSSMYASLGERVTITCKASQDINRFLSWFLQRPGKAPKTLIYRANNLVEGVPSRFSGSGSGQDYSLIISNLEYEDMGIYYCLQYDEFPRTFGGGTKLEIK

SEQ ID NO: 322 - protein, 112 aa, synthetic construct
  source 1..112: note; note (original language) = SB2轻链可变区
DVVMTQTPLTLSITIGQPASISCRSSQSLLDIDGKTYLNWLLQRPGQSPKRLIYLVSELDSGVPDRFTGSGSGTDFTLRISGVEAEDLGIYYCWQGTHFPYTFGGGTKLEIK

SEQ ID NO: 323 - protein, 112 aa, synthetic construct
  source 1..112: note; note (original language) = SB3轻链可变区
DVVMTQTPLTLSITIGQPASISCRSSQSLLDFDGKTYLNWLLQRPGQSPKRLIYLVSELDSGVPDRFTGSGSGTDFTLKISGVEAEDLGIYYCWQGTHFPFTFGGGTKLEIK

SEQ ID NO: 324 - protein, 112 aa, synthetic construct
  source 1..112: note; note (original language) = SB4轻链可变区
DIVMTQAAFSNPVTLGTSASISCRSSRSLLHNNGITYLYWYLQKPGQSPQLLIYQMSNLASGVPDRFHSSGSGTDFTLSISRVEAEDVGVYYCAQNLDLPYTFGGGTKLEIK

SEQ ID NO: 325 - protein, 106 aa, synthetic construct
  source 1..106: note; note (original language) = SB5轻链可变区
QIVLTQSPAIKSASPGEKVTMTCSASSSVIYMHWYQQKSGSSPKRWIYDTSKLASGVPVRFSGSGSGTSYSLTISTMEAEDAATYYCQQWSSYPPTFGGGTKVEIK

SEQ ID NO: 326 - protein, 108 aa, synthetic construct
  source 1..108: note; note (original language) = SB6轻链可变区
SIVMTQTPKFLLVSAGDRVTITCKASQSVNTDVAWYQQKSGQSPKLLIYSASNRYTGVPDRFTGSGYGTDFTFTISTVQAEDLAVYFCQQDHSSPPWTFGGGTKLEIK

SEQ ID NO: 327 - protein, 107 aa, synthetic construct
  source 1..107: note; note (original language) = SB7轻链可变区
DIKMTQSPSSIYVSPGERVTITCKASQDINSFLSWFQQKPGKSPKTLIYRANRLVDGVPSRFSGSGSGQDYSLTISSLEYEDMGIYYCLQYDEFPRTFGGGTKLEIK

SEQ ID NO: 328 - protein, 109 aa, synthetic construct
  source 1..109: note; note (original language) = SB8轻链可变区
QAVVTQESALTTSPGETVTLTCRSSTGAVATSNYANWVQEKPDHLFTGLIGGTNNRVPGVPARFSGSLIGDKAALTITGAQTEDEAIYFCALWYSNHWVFGGGTKLTVL

SEQ ID NO: 329 - protein, 112 aa, synthetic construct
  source 1..112: note; note (original language) = SB9轻链可变区
DVVMTQTPLTLSITIGQPASISCKSSQSLLDSDGKTYLTWLLQRPGQSPKRLIFLVSKLDSGVPDRFTGSGSGTDFTLKISRVEAEDLGVYYCWQGTHFPYTLGGGTKLEIK

SEQ ID NO: 330 - protein, 112 aa, synthetic construct
  source 1..112: note; note (original language) = SB10轻链可变区
DVLMTQTPLSLSVSLGDQASISCRSSQTIVYSNGNSYLEWYLQKPGQSPKLLIYKVSNRFSGIPDRFSGSGSGTDFTLKISRVEAEDLGIYYCFQSSHVPWTFGGGTKLEIK

SEQ ID NO: 331 - protein, 111 aa, synthetic construct
  source 1..111: note; note (original language) = SB11轻链可变区
DIVLTQSPASLAVSLGQRATISCRASQSVSTSSYSYMHWYQLKPGQPPKLLIKYASNLESGVPARFSGSGSGTDFTLNIHPVEEEDAAIYYCQHNWEIPWTFGGGTRLEIK

SEQ ID NO: 332 - protein, 107 aa, synthetic construct
  source 1..107: note; note (original language) = SB12轻链可变区
DVQITQSPSYLAASPGEAITINCRTSKSIGKYLAWYQEKPGKTNKLLIYSGSTLQSGIPSRFSGSGSGTDFTLTITSLEPEDFAMYYCQQHDEYPWTFGGGTKLDIK

SEQ ID NO: 333 - protein, 107 aa, synthetic construct
  source 1..107: note; note (original language) = SB13轻链可变区
DIVMTQSHKFMSTSVGDRVSITCKASQDVSSSVAWYQQKPGQSPKLLIYWASTRHTGVPDRFTGSGSGTDYTLTISSVQAEDLALYYCQQHYNTPPTFGGGTKLEIK

SEQ ID NO: 334 - protein, 109 aa, synthetic construct
  source 1..109: note; note (original language) = SB14轻链可变区
ENVLTQSPAIMSASSGEKVTMTCRASSSVRSSYLHWYQQKSGASPKVWIYSTSNLASGVPVRFSGSGSGTSYSLTISSVEAEDAATYYCQQYSGSPSWTFGGGTKLEIK

SEQ ID NO: 335 - protein, 107 aa, synthetic construct
  source 1..107: note; note (original language) = SB15轻链可变区
DIQMTQSPSSLSASLGERVSLTCRASQEISGYLTWLQQRPDGTIKRLIYAASTLDSGVPKRFSGSRSGSDYSLTISSLESEDFADYYCLQYASYPYTFGGGTKLEIK

SEQ ID NO: 336 - protein, 107 aa, synthetic construct
  source 1..107: note; note (original language) = SB16轻链可变区
DIQMTQSTSSLSASLGDRVTITCRASQDITNYLNWYQQKPDGTVKLLIYYTSRLHSGVPSRFSGSGSGTDFSLTISNLEQEDIATYFCQQGNTLPWTFGGGTKLEII

SEQ ID NO: 337 - protein, 106 aa, synthetic construct
  source 1..106: note; note (original language) = SB17轻链可变区
QIVLTQSPALMTASPGEQVTMTCSASSSVSYIHWYQQKSGTSPKRWIYDASKLASGVPARFSGSGSGTSYSLTISSMEAEDAATYYCQQWSSYPLTFGGGTKLELK

SEQ ID NO: 338 - protein, 107 aa, synthetic construct
  source 1..107: note; note (original language) = SB18轻链可变区
DIQMTQTTSSLSASLGDRVTISCSASQAISNYLNWYQQKPDGTVKLLIYYTSHLHSGVPSRFSGSGSGTDYSLTISNLEPEDIATYYCQQYSKIPWTFGGGTKLEII

SEQ ID NO: 339 - protein, 118 aa, synthetic construct
  source 1..118: note; note (original language) = 人源化抗体3C11重链可变区01
QVQLVQSGAEVKKPGASVKVSCKASGYNFISYWLHWVRQAPGQGLEWMGGIYPGNTDTTYNQKFKGRVTMTRDTSTSTVYMELSSLRSEDTAVYYCIRYDYDRGMDYWGQGTLVTVSS

SEQ ID NO: 340 - protein, 118 aa, synthetic construct
  source 1..118: note; note (original language) = 人源化抗体3C11重链可变区02
QVQLVQSGAEVKKPGASVKVSCKASGYNFISYWLHWVRQAPGQGLEWMGGIYPGNTDTTYNQKFKGRVTMTADTSTSTVYMELSSLRSEDTAVYYCIRYDYDRGMDYWGQGTLVTVSS

SEQ ID NO: 341 - protein, 118 aa, synthetic construct
  source 1..118: note; note (original language) = 人源化抗体3C11重链可变区03
QVQLVQSGAEVKKPGASVKVSCKASGYNFISYWLHWVRQAPGQGLEWMGGIYPGNTDTTYNQKFKGRVTMTADTSTSTAYMELSSLRSEDTAVYYCIRYDYDRGMDYWGQGTLVTVSS

SEQ ID NO: 342 - protein, 118 aa, synthetic construct
  source 1..118: note; note (original language) = 人源化抗体3C11重链可变区04
QVQLVQSGAEVKKPGASVKVSCKASGYNFISYWLHWVRQAPGQGLEWMGGIYPGNTDTTYNQKFKGRVTVTAVTSTSTVYMELSSLRSEDTAVYYCIRYDYDRGMDYWGQGTLVTVSS

SEQ ID NO: 343 - protein, 123 aa, synthetic construct
  source 1..123: note; note (original language) = 人源化抗体8C9重链可变区01
EVQLVESGGGLVQPGRSLRLSCTASGLTFTHYHMSWFRQAPGKGLEWVAIIRNKAYGYTTDYSASVRGRFTISRDDSKSILYLQMNSLKTEDTAVYYCVREGGYGYDGTFAYWGQGTLVTVSS

SEQ ID NO: 344 - protein, 123 aa, synthetic construct
  source 1..123: note; note (original language) = 人源化抗体8C9重链可变区02
EVQLVESGGGLVQPGRSLRLSCTTSGLTFTHYHMSWVRQAPGKGLEWVAIIRNKAYGYTTDYSASVRGRFTISRDDSKSILYLQMNSLKTEDTAVYYCVREGGYGYDGTFAYWGQGTLVTVSS

SEQ ID NO: 345 - protein, 123 aa, synthetic construct
  source 1..123: note; note (original language) = 人源化抗体8C9重链可变区03
EVQLVESGGGLVQPGRSLRLSCTTSGLTFTHYHMSWVRQAPGKGPEWVAIIRNKAYGYTTDYSASVRGRFTISRDDSKSILYLQMNSLKTEDTAVYYCVREGGYGYDGTFAYWGQGTLVTVSS

SEQ ID NO: 346 - protein, 123 aa, synthetic construct
  source 1..123: note; note (original language) = 人源化抗体8C9重链可变区04
EVQLVESGGGLVQPGRSLRLSCTTSGLTFTHYHMSWVRQPPGKAPEWVAIIRNKAYGYTTDYSASVRGRFTISRDDSKSILYLQMNSLKTEDTAVYYCVREGGYGYDGTFAYWGQGTLVTVSS

SEQ ID NO: 347 - protein, 119 aa, synthetic construct
  source 1..119: note; note (original language) = 人源化抗体8E5重链可变区01
QVQLVQSGSELKKPGASVKVSCKASGYTLTDFSMHWVRQAPGQGLEWMGWINTETGAPTYADDFKGRFVFSLDTSVSTAYLQISSLKAEDTAVYYCSRGRDYDPHFDYWGQGTLVTVSS

SEQ ID NO: 348 - protein, 119 aa, synthetic construct
  source 1..119: note; note (original language) = 人源化抗体8E5重链可变区02
QVQLVQSGSELKKPGASVKVSCKASGYTLTDFSMHWVRQAPGQGLEWMGWINTETGAPTYADDFKGRFVLSLDTSVSTAYLQISSLKAEDTAVYYCSRGRDYDPHFDYWGQGTLVTVSS

SEQ ID NO: 349 - protein, 119 aa, synthetic construct
  source 1..119: note; note (original language) = 人源化抗体8E5重链可变区03
QVQLVQSGSELKKPGESVKVSCKASGYTLTDFSMHWVRQAPGQGLEWMGWINTETGAPTYADDFKGRFVLSLDTSVSTAYLQISSLKSEDTAVYYCSRGRDYDPHFDYWGQGTLVTVSS

SEQ ID NO: 350 - protein, 119 aa, synthetic construct
  source 1..119: note; note (original language) = 人源化抗体8E5重链可变区04
QVQLQQSGSELKKPGESVKLSCKASGYTLTDFSMHWVRQAPGQGLKWMGWINTETGAPTYADDFKGRFVFSLDTSVSMAYLQISSLKSEDTAVYYCSRGRDYDPHFDYWGQGTLVTVSS

SEQ ID NO: 351 - protein, 107 aa, synthetic construct
  source 1..107: note; note (original language) = 人源化抗体3C11轻链可变区01
DIQMTQSPSSLSASVGDRVTITCRASEDIYYRLAWYQQKPGKAPKLLISGATALETGVPSRFSGSGSGKDYTFTISSLQPEDIATYYCQHYWNIPWTFGQGTKVEIK

SEQ ID NO: 352 - protein, 107 aa, synthetic construct
  source 1..107: note; note (original language) = 人源化抗体3C11轻链可变区02
DIQMTQSPSSLSASVGDRVTITCRASEDIYYRLAWYQQKPGKAPKLLISGATALETGVPSRFSGSGSGKDYTLTISSLQPEDIATYYCQHYWNIPWTFGQGTKVEIK

SEQ ID NO: 353 - protein, 107 aa, synthetic construct
  source 1..107: note; note (original language) = 人源化抗体3C11轻链可变区03
DIQMTQSPSSLSASVGDRVTITCRASEDIYYRLAWYQQKPGNAPKLLISGATALETGVPSRFSGSGSGKDYTLTISSLQPEDIATYYCQHYWNIPWTFGQGTKVEIK

SEQ ID NO: 354 - protein, 111 aa, synthetic construct
  source 1..111: note; note (original language) = 人源化抗体8C9轻链可变区01
DIQMTQSPSSLSASVGDRVTITCRASESVDNYGISFMNWFQQKPGQAPKLLIYAASNQGSGVPSRFSGSGSGTDFTLTISSMQPEDFATYYCQQSKEVPRTFGGGTKVEIK

SEQ ID NO: 355 - protein, 111 aa, synthetic construct
  source 1..111: note; note (original language) = 人源化抗体8C9轻链可变区02
DIQMTQSPSSLSASVGDRVTITCRASESVDNYGISFMNWFQQKPGQPPKLLIYAASNQGSGVPSRFSGSGSGTDFTLTISSMQPEDFATYYCQQSKEVPRTFGGGTKVEIK

SEQ ID NO: 356 - protein, 111 aa, synthetic construct
  source 1..111: note; note (original language) = 人源化抗体8C9轻链可变区03
DIQMTQSPSSLSASVGDRVTITCRASESVDNYGISFMNWFQQKPGQPPKLLIYAASNQGSGVPSRFSGSGSGTDFTLTISSMQPEDFATYFCQQSKEVPRTFGGGTKVEIK

SEQ ID NO: 357 - protein, 107 aa, synthetic construct
  source 1..107: note; note (original language) = 人源化抗体8E5轻链可变区01
EIVLTQSPATLSLSPGERATLSCRASQSISDFLHWYQQKPGQAPRLLIKYASQSISGIPARFSGSGPGSDFTLTISSVEPEDFAVYYCQSAHSFPYTFGQGTKLEIK

SEQ ID NO: 358 - protein, 107 aa, synthetic construct
  source 1..107: note; note (original language) = 人源化抗体8E5轻链可变区02
EIVLTQSPATLSLSPGERATLSCRASQSISDFLHWYQQKPGQSPRLLIKYASQSISGIPARFSGSGSGSDFTLTISSVEPEDFAVYYCQSAHSFPYTFGQGTKLEIK

SEQ ID NO: 359 - protein, 107 aa, synthetic construct
  source 1..107: note; note (original language) = 人源化抗体8E5轻链可变区03
EIVLTQSPATLSLSPGERATLSCRASQSISDFLHWYQQKSGQSPRLLIKYASQSISGIPARFSGSGSGSDFTLTISSVEPEDFAVYYCQSAHSFPYTFGQGTKLEIK

SEQ ID NO: 360 - protein, 330 aa, synthetic construct
  source 1..330: note; note (original language) = 人IgG1重链恒定区
ASTKGPSVFPLAPSSKSTSGGTAALGCLVKDYFPEPVTVSWNSGALTSGVHTFPAVLQSSGLYSLSSVVTVPSSSLGTQTYICNVNHKPSNTKVDKKVEPKSCDKTHTCPPCPAPELLGGPSVFLFPPKPKDTLMISRTPEVTCVVVDVSHEDPEVKFNWYVDGVEVHNAKTKPREEQYNSTYRVVSVLTVLHQDWLNGKEYKCKVSNKALPAPIEKTISKAKGQPREPQVYTLPPSREEMTKNQVSLTCLVKGFYPSDIAVEWESNGQPENNYKTTPPVLDSDGSFFLYSKLTVDKSRWQQGNVFSCSVMHEALHNHYTQKSLSLSPGK

SEQ ID NO: 361 - protein, 107 aa, synthetic construct [sequence omitted]

SEQ ID NO: 362 - protein, 5 aa, synthetic construct
  source 1..5: note = Kabat 3C11 CDR-H1
SYWLH

SEQ ID NO: 363 - protein, 17 aa, synthetic construct
  source 1..17: note = Kabat 3C11 CDR-H2
GIYPGNTDTTYNQKFKG

SEQ ID NO: 364 - protein, 9 aa, synthetic construct
  source 1..9: note = Kabat/AbM/Chothia 3C11 CDR-H3
YDYDRGMDY

SEQ ID NO: 365 - protein, 11 aa, synthetic construct
  source 1..11: note = Kabat/AbM/Chothia 3C11 CDR-L1
RASEDIYYRLA

SEQ ID NO: 366 - protein, 7 aa, synthetic construct
  source 1..7: note = Kabat/AbM/Chothia 3C11 CDR-L2
GATALET

SEQ ID NO: 367 - protein, 10 aa, synthetic construct
  source 1..10: note = AbM 3C11 CDR-H1
GYNFISYWLH

SEQ ID NO: 368 - protein, 10 aa, synthetic construct
  source 1..10: note = AbM 3C11 CDR-H2
GIYPGNTDTT

SEQ ID NO: 369 - protein, 7 aa, synthetic construct
  source 1..7: note = Chothia 3C11 CDR-H1
GYNFISY

SEQ ID NO: 370 - protein, 6 aa, synthetic construct
  source 1..6: note = Chothia 3C11 CDR-H2
YPGNTD

SEQ ID NO: 371 - protein, 6 aa, synthetic construct
  source 1..6: note = Contact 3C11 CDR-H1
ISYWLH

SEQ ID NO: 372 - protein, 13 aa, synthetic construct
  source 1..13: note = Contact 3C11 CDR-H2
WIGGIYPGNTDTT

SEQ ID NO: 373 - protein, 10 aa, synthetic construct
  source 1..10: note = Contact 3C11 CDR-H3
IRYDYDRGMD

SEQ ID NO: 374 - protein, 7 aa, synthetic construct
  source 1..7: note = Contact 3C11 CDR-L1
YYRLAWY

SEQ ID NO: 375 - protein, 10 aa, synthetic construct
  source 1..10: note = Contact 3C11 CDR-L2
LLISGATALE

SEQ ID NO: 376 - protein, 8 aa, synthetic construct
  source 1..8: note = Contact 3C11 CDR-L3
QHYWNIPW

SEQ ID NO: 377 - protein, 5 aa, synthetic construct
  source 1..5: note = Kabat 8E5 CDR-H1
DFSMH

SEQ ID NO: 378 - protein, 17 aa, synthetic construct
  source 1..17: note = Kabat 8E5 CDR-H2
WINTETGAPTYADDFKG

SEQ ID NO: 379 - protein, 10 aa, synthetic construct
  source 1..10: note = Kabat/AbM/Chothia 8E5 CDR-H3
GRDYDPHFDY

SEQ ID NO: 380 - protein, 11 aa, synthetic construct
  source 1..11: note = Kabat/AbM/Chothia 8E5 CDR-L1
RASQSISDFLH

SEQ ID NO: 381 - protein, 7 aa, synthetic construct
  source 1..7: note = Kabat/AbM/Chothia 8E5 CDR-L2
YASQSIS

SEQ ID NO: 382 - protein, 10 aa, synthetic construct
  source 1..10: note = AbM 8E5 CDR-H1
GYTLTDFSMH

SEQ ID NO: 383 - protein, 10 aa, synthetic construct
  source 1..10: note = AbM 8E5 CDR-H2
WINTETGAPT

SEQ ID NO: 384 - protein, 7 aa, synthetic construct
  source 1..7: note = Chothia 8E5 CDR-H1
GYTLTDF

SEQ ID NO: 385 - protein, 6 aa, synthetic construct
  source 1..6: note = Chothia 8E5 CDR-H2
NTETGA

SEQ ID NO: 386 - protein, 6 aa, synthetic construct
  source 1..6: note = Contact 8E5 CDR-H1
TDFSMH

SEQ ID NO: 387 - protein, 13 aa, synthetic construct
  source 1..13: note = Contact 8E5 CDR-H2
WMGWINTETGAPT

SEQ ID NO: 388 - protein, 11 aa, synthetic construct
  source 1..11: note = Contact 8E5 CDR-H3
SRGRDYDPHFD

SEQ ID NO: 389 - protein, 7 aa, synthetic construct
  source 1..7: note = Contact 8E5 CDR-L1
SDFLHWY

SEQ ID NO: 390 - protein, 10 aa, synthetic construct
  source 1..10: note = Contact 8E5 CDR-L2
LLIKYASQSI

SEQ ID NO: 391 - protein, 8 aa, synthetic construct
  source 1..8: note = Contact 8E5 CDR-L3
QSAHSFPY

SEQ ID NO: 392 - protein, 5 aa, synthetic construct
  source 1..5: note = Kabat 8C9 CDR-H1
HYHMS

SEQ ID NO: 393 - protein, 19 aa, synthetic construct
  source 1..19: note = Kabat 8C9 CDR-H2
IIRNKAYGYTTDYSASVRG

SEQ ID NO: 394 - protein, 12 aa, synthetic construct
  source 1..12: note = Kabat/AbM/Chothia 8C9 CDR-H3
EGGYGYDGTFAY

SEQ ID NO: 395 - protein, 15 aa, synthetic construct
  source 1..15: note = Kabat/AbM/Chothia 8C9 CDR-L1
RASESVDNYGISFMN

SEQ ID NO: 396 - protein, 7 aa, synthetic construct
  source 1..7: note = Kabat/AbM/Chothia 8C9 CDR-L2
AASNQGS

SEQ ID NO: 397 - protein, 10 aa, synthetic construct
  source 1..10: note = AbM 8C9 CDR-H1
GLTFTHYHMS

SEQ ID NO: 398 - protein, 12 aa, synthetic construct
  source 1..12: note = AbM 8C9 CDR-H2
IIRNKAYGYTTD

SEQ ID NO: 399 - protein, 7 aa, synthetic construct
  source 1..7: note = Chothia 8C9 CDR-H1
GLTFTHY

SEQ ID NO: 400 - protein, 8 aa, synthetic construct
  source 1..8: note = Chothia 8C9 CDR-H2
RNKAYGYT

SEQ ID NO: 401 - protein, 6 aa, synthetic construct
  source 1..6: note = Contact 8C9 CDR-H1
THYHMS

SEQ ID NO: 402 - protein, 15 aa, synthetic construct
  source 1..15: note = Contact 8C9 CDR-H2
WLAIIRNKAYGYTTD

SEQ ID NO: 403 - protein, 13 aa, synthetic construct
  source 1..13: note = Contact 8C9 CDR-H3
VREGGYGYDGTFA

SEQ ID NO: 404 - protein, 11 aa, synthetic construct
  source 1..11: note = Contact 8C9 CDR-L1
DNYGISFMNWF

SEQ ID NO: 405 - protein, 10 aa, synthetic construct
  source 1..10: note = Contact 8C9 CDR-L2
LLIYAASNQG

SEQ ID NO: 406 - protein, 8 aa, synthetic construct
  source 1..8: note = Contact 8C9 CDR-L3
QQSKEVPR